European Patent Specification EP 3 580 237 B1, published May 14, 2025. Title: FGF21 MIMETIC ANTIBODIES AND USES THEREOF. Applicant: NOVARTIS AG. The sequence listing filed with the application follows.

SEQUENCE LISTING (64 sequences)

SEQ ID NO: 1 - protein, 209 aa, Homo sapiens
MDSDETGFEHSGLWVSVLAGLLLGACQAHPIPDSSPLLQFGGQVRQRYLYTDDAQQTEAHLEIREDGTVGGAADQSPESLLQLKALKPGVIQILGVKTSRFLCQRPDGALYGSLHFDPEACSFRELLLEDGYNVYQSEAHGLPLHLPGNKSPHRDPAPRGPARFLPLPGLPPALPEPPGILAPQPPDVGSSDPLSMVGPSQGRSPSYAS

SEQ ID NO: 2 - DNA, 938 bp, Homo sapiens
ctgtcagctgaggatccagccgaaagaggagccaggcactcaggccacctgagtctactcacctggacaactggaatctggcaccaattctaaaccactcagcttctccgagctcacaccccggagatcacctgaggacccgagccattgatggactcggacgagaccgggttcgagcactcaggactgtgggtttctgtgctggctggtcttctgctgggagcctgccaggcacaccccatccctgactccagtcctctcctgcaattcgggggccaagtccggcagcggtacctctacacagatgatgcccagcagacagaagcccacctggagatcagggaggatgggacggtggggggcgctgctgaccagagccccgaaagtctcctgcagctgaaagccttgaagccgggagttattcaaatcttgggagtcaagacatccaggttcctgtgccagcggccagatggggccctgtatggatcgctccactttgaccctgaggcctgcagcttccgggagctgcttcttgaggacggatacaatgtttaccagtccgaagcccacggcctcccgctgcacctgccagggaacaagtccccacaccgggaccctgcaccccgaggaccagctcgcttcctgccactaccaggcctgccccccgcactcccggagccacccggaatcctggccccccagccccccgatgtgggctcctcggaccctctgagcatggtgggaccttcccagggccgaagccccagctacgcttcctgaagccagaggctgtttactatgacatctcctctttatttattaggttatttatcttatttatttttttatttttcttacttgagataataaagagttccagaggagaaaaaaaaaaaaaaaaaaaaaaaaaaaaaaaaaaaaaaaaaaaaaaaaaaaaa

SEQ ID NO: 3-5 - skipped (3 entries)

SEQ ID NO: 6 - protein, 11 aa, Artificial Sequence
  source: /note="Description of Artificial Sequence: Synthetic peptide"
GYSITSGYTWH

SEQ ID NO: 7 - protein, 16 aa, Artificial Sequence
  source: /note="Description of Artificial Sequence: Synthetic peptide"
YIHYSVYTNYNPSLKS

SEQ ID NO: 8 - protein, 11 aa, Artificial Sequence
  source: /note="Description of Artificial Sequence: Synthetic peptide"
RTTSLERYFDV

SEQ ID NO: 9 - protein, 6 aa, Artificial Sequence
  source: /note="Description of Artificial Sequence: Synthetic peptide"
SGYTWH

SEQ ID NO: 10 - protein, 8 aa, Artificial Sequence
  source: /note="Description of Artificial Sequence: Synthetic peptide"
GYSITSGY

SEQ ID NO: 11 - protein, 5 aa, Artificial Sequence
  source: /note="Description of Artificial Sequence: Synthetic peptide"
HYSVY

SEQ ID NO: 12 - protein, 9 aa, Artificial Sequence
  source: /note="Description of Artificial Sequence: Synthetic peptide"
GYSITSGYT

SEQ ID NO: 13 - protein, 7 aa, Artificial Sequence
  source: /note="Description of Artificial Sequence: Synthetic peptide"
IHYSVYT

SEQ ID NO: 14 - protein, 13 aa, Artificial Sequence
  source: /note="Description of Artificial Sequence: Synthetic peptide"
ARRTTSLERYFDV

SEQ ID NO: 15 - protein, 120 aa, Artificial Sequence
  source: /note="Description of Artificial Sequence: Synthetic polypeptide"
QVQLQESGPGLVKPSQTLSLTCTVSGYSITSGYTWHWIRQHPGKGLEWIGYIHYSVYTNYNPSLKSRVTISRDTSKNQFSLKLSSVTAADTAVYYCARRTTSLERYFDVWGQGTLVTVSS

SEQ ID NO: 16 - DNA, 360 bp, Artificial Sequence
  source: /note="Description of Artificial Sequence: Synthetic polynucleotide"
caagtgcagctgcaggaatctggccctggcctggtcaagcctagccagaccctgtccctgacctgcaccgtgtccggctactccatcacctccggctacacctggcactggatccggcagcaccccggcaagggcctggaatggatcggctacatccactactccgtgtacaccaactacaaccccagcctgaagtccagagtgaccatctcccgggacacctccaagaaccagttctccctgaagctgtcctccgtgaccgccgctgacaccgccgtgtactactgcgccagacggaccacctccctggaacggtacttcgacgtgtggggccagggcaccctggtcaccgtgtcctct

SEQ ID NO: 17 - protein, 450 aa, Artificial Sequence
  source: /note="Description of Artificial Sequence: Synthetic polypeptide"
QVQLQESGPGLVKPSQTLSLTCTVSGYSITSGYTWHWIRQHPGKGLEWIGYIHYSVYTNYNPSLKSRVTISRDTSKNQFSLKLSSVTAADTAVYYCARRTTSLERYFDVWGQGTLVTVSSASTKGPSVFPLAPSSKSTSGGTAALGCLVKDYFPEPVTVSWNSGALTSGVHTFPAVLQSSGLYSLSSVVTVPSSSLGTQTYICNVNHKPSNTKVDKRVEPKSCDKTHTCPPCPAPELLGGPSVFLFPPKPKDTLMISRTPEVTCVVVAVSHEDPEVKFNWYVDGVEVHNAKTKPREEQYNSTYRVVSVLTVLHQDWLNGKEYKCKVSNKALAAPIEKTISKAKGQPREPQVYTLPPSREEMTKNQVSLTCLVKGFYPSDIAVEWESNGQPENNYKTTPPVLDSDGSFFLYSKLTVDKSRWQQGNVFSCSVMHEALHNHYTQKSLSLSPGK

SEQ ID NO: 18 - DNA, 1350 bp, Artificial Sequence
  source: /note="Description of Artificial Sequence: Synthetic polynucleotide"
caagtgcagctgcaggaatctggccctggcctggtcaagcctagccagaccctgtccctgacctgcaccgtgtccggctactccatcacctccggctacacctggcactggatccggcagcaccccggcaagggcctggaatggatcggctacatccactactccgtgtacaccaactacaaccccagcctgaagtccagagtgaccatctcccgggacacctccaagaaccagttctccctgaagctgtcctccgtgaccgccgctgacaccgccgtgtactactgcgccagacggaccacctccctggaacggtacttcgacgtgtggggccagggcaccctggtcaccgtgtcctctgcttccaccaaggggccctccgtgttccctctggccccttccagcaagtccacctctggcggcaccgccgctctgggctgcctcgtgaaggactacttccccgagcccgtgaccgtgtcctggaactctggcgccctgacctccggcgtgcacaccttccctgccgtgctgcagtcctccggcctgtactccctgtccagcgtcgtgaccgtgccctccagctctctgggcacccagacctacatctgcaacgtgaaccacaagccctccaacaccaaagtggacaagcgggtggaacccaagtcctgcgacaagacccacacctgtcctccctgccctgcccctgagctgctgggcggaccttccgtgttcctgttccctccaaagcccaaggacaccctgatgatctcccggacccctgaagtgacctgcgtggtggtggccgtgtcccacgaggatcccgaagtgaagttcaattggtacgtggacggcgtggaagtgcacaacgccaagaccaagcccagagaggaacagtacaactccacctaccgggtggtgtccgtgctgaccgtgctgcaccaggactggctgaacggcaaagagtacaagtgcaaagtgtccaacaaggccctggccgctcccatcgaaaagaccatctccaaggccaagggccagccccgcgagccccaagtgtacacactgcctcccagccgggaagagatgaccaagaatcaagtgtccctgacatgtctggtcaagggcttctaccctagcgatatcgccgtggaatgggagtccaacggccagcctgagaacaactacaagaccacccctcccgtgctggactccgacggctcattcttcctgtactccaagctgaccgtggacaagtcccggtggcagcagggcaacgtgttctcctgctccgtgatgcacgaggccctgcacaaccactacacccagaagtccctgagcctgtcccctggcaag

SEQ ID NO: 19 - protein, 11 aa, Artificial Sequence
  source: /note="Description of Artificial Sequence: Synthetic peptide"
QASQDISNYLN

SEQ ID NO: 20 - protein, 7 aa, Artificial Sequence
  source: /note="Description of Artificial Sequence: Synthetic peptide"
YTSRLQS

SEQ ID NO: 21 - protein, 9 aa, Artificial Sequence
  source: /note="Description of Artificial Sequence: Synthetic peptide"
QQGNTLPYT

SEQ ID NO: 22 - protein, 7 aa, Artificial Sequence
  source: /note="Description of Artificial Sequence: Synthetic peptide"
SQDISNY

SEQ ID NO: 23 - protein, 3 aa, Artificial Sequence
  source: /note="Description of Artificial Sequence: Synthetic peptide"
YTS

SEQ ID NO: 24 - protein, 6 aa, Artificial Sequence
  source: /note="Description of Artificial Sequence: Synthetic peptide"
GNTLPY

SEQ ID NO: 25 - protein, 6 aa, Artificial Sequence
  source: /note="Description of Artificial Sequence: Synthetic peptide"
QDISNY

SEQ ID NO: 26 - protein, 107 aa, Artificial Sequence
  source: /note="Description of Artificial Sequence: Synthetic polypeptide"
DIQMTQSPSSLSASVGDRVTITCQASQDISNYLNWYQQKPGKAPKLLIYYTSRLQSGVPSRFSGSGSGADYTFTISSLQPEDIATYFCQQGNTLPYTFGQGTKLEIK

SEQ ID NO: 27 - DNA, 321 bp, Artificial Sequence
  source: /note="Description of Artificial Sequence: Synthetic polynucleotide"
gacatccagatgacccagagcccgtcgtccctctccgcttccgtgggagatagagtgaccatcacctgtcaagccagccaggatatttcaaactacctgaattggtaccagcagaagccggggaaggctcccaagttgctcatctactacacatcgaggctgcagtccggcgtgcccagccggttctccgggtccggatcaggcgccgactataccttcaccatttcctccctgcaaccggaggacattgccacttacttctgccaacaagggaacaccctgccctacactttcggacaaggaactaagctggaaatcaag

SEQ ID NO: 28 - protein, 214 aa, Artificial Sequence
  source: /note="Description of Artificial Sequence: Synthetic polypeptide"
DIQMTQSPSSLSASVGDRVTITCQASQDISNYLNWYQQKPGKAPKLLIYYTSRLQSGVPSRFSGSGSGADYTFTISSLQPEDIATYFCQQGNTLPYTFGQGTKLEIKRTVAAPSVFIFPPSDEQLKSGTASVVCLLNNFYPREAKVQWKVDNALQSGNSQESVTEQDSKDSTYSLSSTLTLSKADYEKHKVYACEVTHQGLSSPVTKSFNRGEC

SEQ ID NO: 29 - DNA, 642 bp, Artificial Sequence
  source: /note="Description of Artificial Sequence: Synthetic polynucleotide"
gacatccagatgacccagagcccctccagcctgtccgcctccgtgggcgacagagtgaccatcacctgtcaggcctcccaggacatctccaactacctgaactggtatcagcagaagcccggcaaggcccctaagctgctgatctactacacctcccggctgcagtccggcgtgccctccagattctccggctctggctctggcgccgactacaccttcaccatctccagcctgcagcccgaggatatcgctacctacttctgtcagcaaggcaacaccctgccctacaccttcggccagggcaccaagctggaaatcaagcgtacggtggccgctccctccgtgttcatcttcccaccctccgacgagcagctgaagtccggcaccgcctccgtcgtgtgcctgctgaacaacttctaccctcgcgaggccaaagtgcagtggaaagtggacaacgccctgcagagcggcaactcccaggaatccgtcaccgagcaggactccaaggacagcacctactccctgtcctccaccctgaccctgtccaaggccgactacgagaagcacaaagtgtacgcctgcgaagtgacccaccagggcctgtccagccccgtgaccaagtccttcaaccggggcgagtgc

SEQ ID NO: 30 - DNA, 1350 bp, Artificial Sequence; identical to SEQ ID NO: 18
  source: /note="Description of Artificial Sequence: Synthetic polynucleotide"

SEQ ID NO: 31 - protein, 11 aa, Artificial Sequence
  source: /note="Description of Artificial Sequence: Synthetic peptide"
RASQDISNYLN

SEQ ID NO: 32 - protein, 107 aa, Artificial Sequence
  source: /note="Description of Artificial Sequence: Synthetic polypeptide"
EIVMTQSPATLSLSPGERATLSCRASQDISNYLNWYQQKPGQAPRLLIYYTSRLQSGIPARFSGSGSGADYTLTISSLQPEDFAVYFCQQGNTLPYTFGQGTKLEIK

SEQ ID NO: 33 - DNA, 321 bp, Artificial Sequence
  source: /note="Description of Artificial Sequence: Synthetic polynucleotide"
gagatcgtgatgacccagtcccctgccaccctgtccctgagccctggcgagagagccaccctgagctgccgggcctcccaggacatctccaactacctgaactggtatcagcagaagcccggccaggcccctcggctgctgatctactacacctcccggctgcagtccggcatccctgccagattctccggctctggctctggcgccgactacaccctgaccatctccagcctgcagcccgaggacttcgccgtgtacttctgtcagcaaggcaacaccctgccctacaccttcggccagggcaccaagctggaaatcaag

SEQ ID NO: 34 - protein, 214 aa, Artificial Sequence
  source: /note="Description of Artificial Sequence: Synthetic polypeptide"
EIVMTQSPATLSLSPGERATLSCRASQDISNYLNWYQQKPGQAPRLLIYYTSRLQSGIPARFSGSGSGADYTLTISSLQPEDFAVYFCQQGNTLPYTFGQGTKLEIKRTVAAPSVFIFPPSDEQLKSGTASVVCLLNNFYPREAKVQWKVDNALQSGNSQESVTEQDSKDSTYSLSSTLTLSKADYEKHKVYACEVTHQGLSSPVTKSFNRGEC

SEQ ID NO: 35 - DNA, 642 bp, Artificial Sequence
  source: /note="Description of Artificial Sequence: Synthetic polynucleotide"
gagatcgtgatgacccagtcccctgccaccctgtccctgagccctggcgagagagccaccctgagctgccgggcctcccaggacatctccaactacctgaactggtatcagcagaagcccggccaggcccctcggctgctgatctactacacctcccggctgcagtccggcatccctgccagattctccggctctggctctggcgccgactacaccctgaccatctccagcctgcagcccgaggacttcgccgtgtacttctgtcagcaaggcaacaccctgccctacaccttcggccagggcaccaagctggaaatcaagcgtacggtggccgctccctccgtgttcatcttcccaccctccgacgagcagctgaagtccggcaccgcctccgtcgtgtgcctgctgaacaacttctaccctcgcgaggccaaagtgcagtggaaagtggacaacgccctgcagagcggcaactcccaggaatccgtcaccgagcaggactccaaggacagcacctactccctgtcctccaccctgaccctgtccaaggccgactacgagaagcacaaagtgtacgcctgcgaagtgacccaccagggcctgtccagccccgtgaccaagtccttcaaccggggcgagtgc

SEQ ID NO: 36 - DNA, 360 bp, Artificial Sequence
  source: /note="Description of Artificial Sequence: Synthetic polynucleotide"
caagtccagctgcaagaatccggacccggcctcgtcaagccgtcccagactctgtctctcacttgcacggtgtcaggctacagcatcaccagcggttacacctggcactggatcaggcagcatcctggaaaggggctggaatggattgggtacattcactactcggtgtacaccaactacaacccatcgctcaagtcgagagtcaccatttcccgggacacctccaagaaccagttcagcctcaagctgtcctctgtgaccgccgctgatactgccgtgtactattgcgcacgccggactacttccctggagcgctacttcgacgtctggggccagggcactttggtcaccgtcagctcc

SEQ ID NO: 37 - DNA, 1350 bp, Artificial Sequence
  source: /note="Description of Artificial Sequence: Synthetic polynucleotide"
caagtccagctgcaagaatccggacccggcctcgtcaagccgtcccagactctgtctctcacttgcacggtgtcaggctacagcatcaccagcggttacacctggcactggatcaggcagcatcctggaaaggggctggaatggattgggtacattcactactcggtgtacaccaactacaacccatcgctcaagtcgagagtcaccatttcccgggacacctccaagaaccagttcagcctcaagctgtcctctgtgaccgccgctgatactgccgtgtactattgcgcacgccggactacttccctggagcgctacttcgacgtctggggccagggcactttggtcaccgtcagctccgccagcactaagggccccagcgtgtttccgctggccccctcctccaaaagcacctccggcggaactgccgcgctcggatgtctcgtgaaggactatttccccgagcctgtgacagtgtcatggaactcgggagcactgaccagcggagtgcatacttttcccgcggtcctgcagtcctccggattgtacagcctgtcatcggtcgtgaccgtgccgtcctcatcgctgggcacccagacctacatctgcaacgtgaaccacaaacctagcaacaccaaagtggataagcgggtggaacctaagtcctgcgacaagactcacacttgtccgccatgcccagcgcctgaactcctgggtggtccttcggtgttcctgttcccgccaaagccgaaggacaccctgatgatctcccggacgcctgaagtgacctgtgtggtggtggctgtgtcacatgaggaccctgaagtcaagttcaattggtacgtggacggcgtggaggtgcacaacgccaagaccaagcctagagaggaacagtacaactccacctaccgcgtcgtgtcggtgctgaccgtgttgcaccaagactggctgaatggaaaggagtataagtgcaaagtgtccaacaaggccctggccgcaccaattgagaaaaccatctccaaggccaagggacagccgcgcgaaccccaagtgtacacccttcccccgtcccgggaggaaatgaccaagaatcaagtctccctgacttgccttgtgaagggtttctacccctccgacatcgccgtggagtgggagtcaaacgggcagccggaaaacaactacaagaccacacctccggtgctggattccgacggctccttcttcttgtactcgaagctgaccgtggataagagcaggtggcagcagggaaacgtgttctcctgctccgtgatgcacgaagctctgcacaaccactacactcagaagtcgctctcgctgagccccgggaag

SEQ ID NO: 38 - DNA, 360 bp, Artificial Sequence; identical to SEQ ID NO: 36
  source: /note="Description of Artificial Sequence: Synthetic polynucleotide"

SEQ ID NO: 39 - DNA, 1350 bp, Artificial Sequence; identical to SEQ ID NO: 37
  source: /note="Description of Artificial Sequence: Synthetic polynucleotide"

SEQ ID NO: 40 - DNA, 321 bp, Artificial Sequence
  source: /note="Description of Artificial Sequence: Synthetic polynucleotide"
gaaatcgtgatgactcagtcccccgccactctctccctgtcccctggcgaacgggccaccctgtcgtgccgggcgtcgcaggacatctcaaactatctgaactggtaccagcagaagcctggacaggcacccaggctcctgatctactacacctcgcgcctgcaatccggaatcccagcccgcttctccggttccggctccggcgctgattacaccctcaccattagcagcctgcagccggaggacttcgccgtgtacttctgtcaacaaggaaacaccctcccgtacacatttgggcagggaaccaagctggagattaag

SEQ ID NO: 41 - DNA, 642 bp, Artificial Sequence
  source: /note="Description of Artificial Sequence: Synthetic polynucleotide"
gaaatcgtgatgactcagtcccccgccactctctccctgtcccctggcgaacgggccaccctgtcgtgccgggcgtcgcaggacatctcaaactatctgaactggtaccagcagaagcctggacaggcacccaggctcctgatctactacacctcgcgcctgcaatccggaatcccagcccgcttctccggttccggctccggcgctgattacaccctcaccattagcagcctgcagccggaggacttcgccgtgtacttctgtcaacaaggaaacaccctcccgtacacatttgggcagggaaccaagctggagattaagcgtacggtggccgcgccgtccgtgttcatcttccctccttctgacgagcagctcaagagcggcaccgcgtcggtggtctgcctgctgaacaacttctacccacgggaggccaaggtccagtggaaagtggataacgcattgcagtcgggaaactcacaggagtcggtgaccgaacaggactccaaagactcaacctactccctgtcctccactcttaccctgtccaaggcggactacgaaaagcacaaggtctacgcctgcgaagtgacccatcagggtctgagcagccctgtgactaagagctttaaccgcggcgaatgc

SEQ ID NO: 42 - protein, 16 aa, Artificial Sequence
  source: /note="Description of Artificial Sequence: Synthetic peptide"
YIHYSVYTNYNPSVKG

SEQ ID NO: 43 - protein, 120 aa, Artificial Sequence
  source: /note="Description of Artificial Sequence: Synthetic polypeptide"
EVQLVESGGGLVKPGGSLRLSCAVSGYSITSGYTWHWVRQAPGKGLEWLSYIHYSVYTNYNPSVKGRFTISRDTAKNSFYLQMNSLRAEDTAVYYCARRTTSLERYFDVWGQGTLVTVSS

SEQ ID NO: 44 - DNA, 360 bp, Artificial Sequence
  source: /note="Description of Artificial Sequence: Synthetic polynucleotide"
gaagtccaactcgtcgaatccggcggcggactggtcaagccgggaggatcgctgagactgtcgtgcgcagtgtcagggtacagcatcacctccggttacacctggcactgggtcagacaggcgccgggaaaaggcctggaatggctgtcctacattcattactccgtgtacactaactacaacccctcagtgaaggggcggttcaccatctcccgggacactgccaagaatagcttctatctgcaaatgaactccctgcgggccgaggataccgccgtgtactactgcgcgaggcgcaccacgtccctggagcgctactttgacgtgtggggccagggtaccctcgtgactgtgtcctcg

SEQ ID NO: 45 - protein, 450 aa, Artificial Sequence
  source: /note="Description of Artificial Sequence: Synthetic polypeptide"
EVQLVESGGGLVKPGGSLRLSCAVSGYSITSGYTWHWVRQAPGKGLEWLSYIHYSVYTNYNPSVKGRFTISRDTAKNSFYLQMNSLRAEDTAVYYCARRTTSLERYFDVWGQGTLVTVSSASTKGPSVFPLAPSSKSTSGGTAALGCLVKDYFPEPVTVSWNSGALTSGVHTFPAVLQSSGLYSLSSVVTVPSSSLGTQTYICNVNHKPSNTKVDKRVEPKSCDKTHTCPPCPAPELLGGPSVFLFPPKPKDTLMISRTPEVTCVVVAVSHEDPEVKFNWYVDGVEVHNAKTKPREEQYNSTYRVVSVLTVLHQDWLNGKEYKCKVSNKALAAPIEKTISKAKGQPREPQVYTLPPSREEMTKNQVSLTCLVKGFYPSDIAVEWESNGQPENNYKTTPPVLDSDGSFFLYSKLTVDKSRWQQGNVFSCSVMHEALHNHYTQKSLSLSPGK

SEQ ID NO: 46 - DNA, 1350 bp, Artificial Sequence
  source: /note="Description of Artificial Sequence: Synthetic polynucleotide"
gaagtccaactcgtcgaatccggcggcggactggtcaagccgggaggatcgctgagactgtcgtgcgcagtgtcagggtacagcatcacctccggttacacctggcactgggtcagacaggcgccgggaaaaggcctggaatggctgtcctacattcattactccgtgtacactaactacaacccctcagtgaaggggcggttcaccatctcccgggacactgccaagaatagcttctatctgcaaatgaactccctgcgggccgaggataccgccgtgtactactgcgcgaggcgcaccacgtccctggagcgctactttgacgtgtggggccagggtaccctcgtgactgtgtcctcggctagcaccaagggcccctccgtgttccctctggccccttccagcaagtctacctccggcggcacagctgctctgggctgcctggtcaaggactacttccctgagcctgtgacagtgtcctggaactctggcgccctgacctctggcgtgcacaccttccctgccgtgctgcagtcctccggcctgtactccctgtcctccgtggtcacagtgccttcaagcagcctgggcacccagacctatatctgcaacgtgaaccacaagccttccaacaccaaggtggacaagcgggtggagcctaagtcctgcgacaagacccacacctgtcctccctgccctgctcctgaactgctgggcggcccttctgtgttcctgttccctccaaagcccaaggacaccctgatgatctcccggacccctgaagtgacctgcgtggtggtggccgtgtcccacgaggatcctgaagtgaagttcaattggtacgtggacggcgtggaggtgcacaacgccaagaccaagcctcgggaggaacagtacaactccacctaccgggtggtgtccgtgctgaccgtgctgcaccaggactggctgaacggcaaagagtacaagtgcaaagtctccaacaaggccctggccgcccctatcgaaaagacaatctccaaggccaagggccagcctagggaaccccaggtgtacaccctgccacccagccgggaggaaatgaccaagaaccaggtgtccctgacctgtctggtcaagggcttctacccttccgatatcgccgtggagtgggagtctaacggccagcctgagaacaactacaagaccacccctcctgtgctggactccgacggctccttcttcctgtactccaaactgaccgtggacaagtcccggtggcagcagggcaacgtgttctcctgctccgtgatgcacgaggccctgcacaaccactacacccagaagtccctgtccctgtctcccggcaag

SEQ ID NO: 47 - protein, 107 aa, Artificial Sequence
  source: /note="Description of Artificial Sequence: Synthetic polypeptide"
DIQMTQSPSSLSASVGDRVTITCQASQDISNYLNWYQQKPGKAPKLLIYYTSRLQSGVPSRFTGSGSGADYTFTISSLQPEDIATYFCQQGNTLPYTFGQGTKLEIK

SEQ ID NO: 48 - DNA, 321 bp, Artificial Sequence
  source: /note="Description of Artificial Sequence: Synthetic polynucleotide"
gatattcagatgactcagagcccctcctcgctctccgcctccgtgggggatcgcgtgacaatcacctgtcaagcgtcccaggacatctcaaactacctgaactggtatcagcagaagccagggaaggccccgaagctgctgatctactacacttcgcggctgcagtccggcgtgccgtcacggttcactggctcgggctccggagcagactacaccttcaccattagcagcctgcagcccgaggacatcgctacctacttttgccaacaaggaaacaccctgccttacaccttcggacagggtactaagctggaaatcaaa

SEQ ID NO: 49 - protein, 214 aa, Artificial Sequence
  source: /note="Description of Artificial Sequence: Synthetic polypeptide"
DIQMTQSPSSLSASVGDRVTITCQASQDISNYLNWYQQKPGKAPKLLIYYTSRLQSGVPSRFTGSGSGADYTFTISSLQPEDIATYFCQQGNTLPYTFGQGTKLEIKRTVAAPSVFIFPPSDEQLKSGTASVVCLLNNFYPREAKVQWKVDNALQSGNSQESVTEQDSKDSTYSLSSTLTLSKADYEKHKVYACEVTHQGLSSPVTKSFNRGEC

SEQ ID NO: 50 - DNA, 642 bp, Artificial Sequence
  source: /note="Description of Artificial Sequence: Synthetic polynucleotide"
gatattcagatgactcagagcccctcctcgctctccgcctccgtgggggatcgcgtgacaatcacctgtcaagcgtcccaggacatctcaaactacctgaactggtatcagcagaagccagggaaggccccgaagctgctgatctactacacttcgcggctgcagtccggcgtgccgtcacggttcactggctcgggctccggagcagactacaccttcaccattagcagcctgcagcccgaggacatcgctacctacttttgccaacaaggaaacaccctgccttacaccttcggacagggtactaagctggaaatcaaacgtacggtggccgctcccagcgtgttcatcttcccccccagcgacgagcagctgaagagcggcaccgccagcgtggtgtgcctgctgaacaacttctacccccgggaggccaaggtgcagtggaaggtggacaacgccctgcagagcggcaacagccaggagagcgtcaccgagcaggacagcaaggactccacctacagcctgagcagcaccctgaccctgagcaaggccgactacgagaagcataaggtgtacgcctgcgaggtgacccaccagggcctgtccagccccgtgaccaagagcttcaacaggggcgagtgc

SEQ ID NO: 51 - DNA, 642 bp, Artificial Sequence
  source: /note="Description of Artificial Sequence: Synthetic polynucleotide"
gacatccagatgacccagagcccgtcgtccctctccgcttccgtgggagatagagtgaccatcacctgtcaagccagccaggatatttcaaactacctgaattggtaccagcagaagccggggaaggctcccaagttgctcatctactacacatcgaggctgcagtccggcgtgcccagccggttctccgggtccggatcaggcgccgactataccttcaccatttcctccctgcaaccggaggacattgccacttacttctgccaacaagggaacaccctgccctacactttcggacaaggaactaagctggaaatcaagcgtacggtggccgcgccgtccgtgttcatcttccctccttctgacgagcagctcaagagcggcaccgcgtcggtggtctgcctgctgaacaacttctacccacgggaggccaaggtccagtggaaagtggataacgcattgcagtcgggaaactcacaggagtcggtgaccgaacaggactccaaagactcaacctactccctgtcctccactcttaccctgtccaaggcggactacgaaaagcacaaggtctacgcctgcgaagtgacccatcagggtctgagcagccctgtgactaagagctttaaccgcggcgaatgc

SEQ ID NO: 52 - protein, 1044 aa, Homo sapiens
MKPGCAAGSPGNEWIFFSTDEITTRYRNTMSNGGLQRSVILSALILLRAVTGFSGDGRAIWSKNPNFTPVNESQLFLYDTFPKNFFWGIGTGALQVEGSWKKDGKGPSIWDHFIHTHLKNVSSTNGSSDSYIFLEKDLSALDFIGVSFYQFSISWPRLFPDGIVTVANAKGLQYYSTLLDALVLRNIEPIVTLYHWDLPLALQEKYGGWKNDTIIDIFNDYATYCFQMFGDRVKYWITIHNPYLVAWHGYGTGMHAPGEKGNLAAVYTVGHNLIKAHSKVWHNYNTHFRPHQKGWLSITLGSHWIEPNRSENTMDIFKCQQSMVSVLGWFANPIHGDGDYPEGMRKKLFSVLPIFSEAEKHEMRGTADFFAFSFGPNNFKPLNTMAKMGQNVSLNLREALNWIKLEYNNPRILIAENGWFTDSRVKTEDTTAIYMMKNFLSQVLQAIRLDEIRVFGYTAWSLLDGFEWQDAYTIRRGLFYVDFNSKQKERKPKSSAHYYKQIIRENGFSLKESTPDVQGQFPCDFSWGVTESVLKPESVASSPQFSDPHLYVWNATGNRLLHRVEGVRLKTRPAQCTDFVNIKKQLEMLARMKVTHYRFALDWASVLPTGNLSAVNRQALRYYRCVVSEGLKLGISAMVTLYYPTHAHLGLPEPLLHADGWLNPSTAEAFQAYAGLCFQELGDLVKLWITINEPNRLSDIYNRSGNDTYGAAHNLLVAHALAWRLYDRQFRPSQRGAVSLSLHADWAEPANPYADSHWRAAERFLQFEIAWFAEPLFKTGDYPAAMREYIASKHRRGLSSSALPRLTEAERRLLKGTVDFCALNHFTTRFVMHEQLAGSRYDSDRDIQFLQDITRLSSPTRLAVIPWGVRKLLRWVRRNYGDMDIYITASGIDDQALEDDRLRKYYLGKYLQEVLKAYLIDKVRIKGYYAFKLAEEKSKPRFGFFTSDFKAKSSIQFYNKVISSRGFPFENSSSRCSQTQENTECTVCLFLVQKKPLIFLGCCFFSTLVLLLSIAIFQRQKRRKFWKAKNLQHIPLKKGKRVVS

SEQ ID NO: 53 - protein, 181 aa, Homo sapiens
HPIPDSSPLLQFGGQVRQRYLYTDDAQQTEAHLEIREDGTVGGAADQSPESLLQLKALKPGVIQILGVKTSRFLCQRPDGALYGSLHFDPEACSFRELLLEDGYNVYQSEAHGLPLHLPGNKSPHRDPAPRGPARFLPLPGLPPALPEPPGILAPQPPDVGSSDPLSMVGPSQGRSPSYAS

SEQ ID NO: 54 - DNA, 321 bp, Artificial Sequence
  source: /note="Description of Artificial Sequence: Synthetic polynucleotide"
gacatccagatgacccagagcccctccagcctgtccgcctccgtgggcgacagagtgaccatcacctgtcaggcctcccaggacatctccaactacctgaactggtatcagcagaagcccggcaaggcccctaagctgctgatctactacacctcccggctgcagtccggcgtgccctccagattctccggctctggctctggcgccgactacaccttcaccatctccagcctgcagcccgaggatatcgctacctacttctgtcagcaaggcaacaccctgccctacaccttcggccagggcaccaagctggaaatcaag

SEQ ID NO: 55 - protein, 119 aa, Artificial Sequence
  source: /note="Description of Artificial Sequence: Synthetic polypeptide"
QVQLVQSGAEVKKPGSSVKVSCKASGYTFTDYYINWVRQAPGQGLEWMGRIHPGSGNTYYNEKFQGRVTLTADKSTSTAYMELSSLRSEDTAVYYCAILLLRSYGMDDWGQGTTVTVSS

SEQ ID NO: 56 - protein, 449 aa, Artificial Sequence
  source: /note="Description of Artificial Sequence: Synthetic polypeptide"
QVQLVQSGAEVKKPGSSVKVSCKASGYTFTDYYINWVRQAPGQGLEWMGRIHPGSGNTYYNEKFQGRVTLTADKSTSTAYMELSSLRSEDTAVYYCAILLLRSYGMDDWGQGTTVTVSSASTKGPSVFPLAPSSKSTSGGTAALGCLVKDYFPEPVTVSWNSGALTSGVHTFPAVLQSSGLYSLSSVVTVPSSSLGTQTYICNVNHKPSNTKVDKRVEPKSCDKTHTCPPCPAPEAAGGPSVFLFPPKPKDTLMISRTPEVTCVVVDVSHEDPEVKFNWYVDGVEVHNAKTKPREEQYNSTYRVVSVLTVLHQDWLNGKEYKCKVSNKALPAPIEKTISKAKGQPREPQVYTLPPSREEMTKNQVSLTCLVKGFYPSDIAVEWESNGQPENNYKTTPPVLDSDGSFFLYSKLTVDKSRWQQGNVFSCSVMHEALHNHYTQKSLSLSPGK

SEQ ID NO: 57 - protein, 112 aa, Artificial Sequence
  source: /note="Description of Artificial Sequence: Synthetic polypeptide"
DVVMTQTPLSLSVTPGQPASISCKSSQSIVHSSGNTYLEWYLQKPGQSPQLLIYKVSNRFSGVPDRFSGSGSGTDFTLKISRVEAEDVGVYYCFQGSHIPYTFGQGTKLEIK

SEQ ID NO: 58 - protein, 219 aa, Artificial Sequence
  source: /note="Description of Artificial Sequence: Synthetic polypeptide"
DVVMTQTPLSLSVTPGQPASISCKSSQSIVHSSGNTYLEWYLQKPGQSPQLLIYKVSNRFSGVPDRFSGSGSGTDFTLKISRVEAEDVGVYYCFQGSHIPYTFGQGTKLEIKRTVAAPSVFIFPPSDEQLKSGTASVVCLLNNFYPREAKVQWKVDNALQSGNSQESVTEQDSKDSTYSLSSTLTLSKADYEKHKVYACEVTHQGLSSPVTKSFNRGEC

SEQ ID NO: 59 - protein, 450 aa, Artificial Sequence
  source: /note="Description of Artificial Sequence: Synthetic polypeptide"
EVQLVESGGGLVKPGGSLRLSCAVSGYSITSGYTWHWVRQAPGKGLEWLSYIHYSVYTNYNPSVKGRFTISRDTAKNSFYLQMNSLRAEDTAVYYCARRTTSLERYFDVWGQGTLVTVSSASTKGPSVFPLAPSSKSTSGGTAALGCLVKDYFPEPVTVSWNSGALTSGVHTFPAVLQSSGLYSLSSVVTVPSSSLGTQTYICNVNHKPSNTKVDKRVEPKSCDKTHTCPPCPAPEAAGGPSVFLFPPKPKDTLMISRTPEVTCVVVDVSHEDPEVKFNWYVDGVEVHNAKTKPREEQYNSTYRVVSVLTVLHQDWLNGKEYKCKVSNKALPAPIEKTISKAKGQPREPQVYTLPPSREEMTKNQVSLTCLVKGFYPSDIAVEWESNGQPENNYKTTPPVLDSDGSFFLYSKLTVDKSRWQQGNVFSCSVMHEALHNHYTQKSLSLSPGK

SEQ ID NO: 60 - protein, 214 aa, Artificial Sequence; identical to SEQ ID NO: 49
  source: /note="Description of Artificial Sequence: Synthetic polypeptide"

SEQ ID NO: 61 - protein, 449 aa, Artificial Sequence
  source: /note="Description of Artificial Sequence: Synthetic polypeptide"
QVQLVQSGAEVKKPGSSVKVSCKASGYTFTDYYINWVRQAPGQGLEWMGRIHPGSGNTYYNEKFQGRVTLTADKSTSTAYMELSSLRSEDTAVYYCAILLLRSYGMDDWGQGTTVTVSSASTKGPSVFPLAPSSKSTSGGTAALGCLVKDYFPEPVTVSWNSGALTSGVHTFPAVLQSSGLYSLSSVVTVPSSSLGTQTYICNVNHKPSNTKVDKRVEPKSCDKTHTCPPCPAPELLGGPSVFLFPPKPKDTLMISRTPEVTCVVVAVSHEDPEVKFNWYVDGVEVHNAKTKPREEQYNSTYRVVSVLTVLHQDWLNGKEYKCKVSNKALAAPIEKTISKAKGQPREPQVYTLPPSREEMTKNQVSLTCLVKGFYPSDIAVEWESNGQPENNYKTTPPVLDSDGSFFLYSKLTVDKSRWQQGNVFSCSVMHEALHNHYTQKSLSLSPGK

SEQ ID NO: 62 - protein, 219 aa, Artificial Sequence; identical to SEQ ID NO: 58
  source: /note="Description of Artificial Sequence: Synthetic polypeptide"

SEQ ID NO: 63 - DNA, 546 bp, Homo sapiens
caccccatccctgactccagtcctctcctgcaattcgggggccaagtccggcagcggtacctctacacagatgatgcccagcagacagaagcccacctggagatcagggaggatgggacggtggggggcgctgctgaccagagccccgaaagtctcctgcagctgaaagccttgaagccgggagttattcaaatcttgggagtcaagacatccaggttcctgtgccagcggccagatggggccctgtatggatcgctccactttgaccctgaggcctgcagcttccgggagctgcttcttgaggacggatacaatgtttaccagtccgaagcccacggcctcccgctgcacctgccagggaacaagtccccacaccgggaccctgcaccccgaggaccagctcgcttcctgccactaccaggcctgccccccgcactcccggagccacccggaatcctggccccccagccccccgatgtgggctcctcggaccctctgagcatggtgggaccttcccagggccgaagccccagctacgcttcctga

SEQ ID NO: 64 - protein, 6 aa, Artificial Sequence
  source: /note="Description of Artificial Sequence: Synthetic 6xHis tag"
HHHHHH